European Patent Specification EP 3 431 095 B1, published November 1, 2023. Title: Cyclotides as immunosuppressive agents. Applicant: Medizinische Universität Wien et al. The sequence listing filed with the application follows.

SEQUENCE LISTING (17 sequences)

SEQ ID NO: 1 - protein, 29 aa, Oldenlandia affinis
GLPVCGETCVGGTCNTPGCTCSWPVCTRN

SEQ ID NO: 2 - protein, 29 aa, Oldenlandia affinis
GLPVCGETCFGGTCNTPGCSCTWPICTRD

SEQ ID NO: 3 - protein, 29 aa, Artificial Sequence
  Mutant form of Kalata B1
GLPVCGETCFGGTCNTPGCSCTWPICTRD

SEQ ID NO: 4 - protein, 29 aa, Artificial Sequence
  Mutant form of Kalata B1
GLPVCGETCVGGTCNTPKCTCSWPVCTRN

SEQ ID NO: 5 - protein, 29 aa, Artificial Sequence
  Mutant form of Kalata B1
GLPVCGETCVGGTCNTPGCTCSWPVCTRK

SEQ ID NO: 6 - protein, 29 aa, Artificial Sequence
  Mutant form of Kalata B1
KLPVCGETCVGGTCNTPGCKCSWPVCTRN

SEQ ID NO: 7 - protein, 29 aa, Artificial Sequence
  Mutant form of Kalata B1
GLPVCGETCVGGTCNTPGCKCSWPVCTRN

SEQ ID NO: 8 - protein, 29 aa, Artificial Sequence
  Mutant form of Kalata B1
GLPVCGEKCVGGTCNTPGCTCSWPVCTRN

SEQ ID NO: 9 - protein, 29 aa, Artificial Sequence
  Mutant form of Kalata B1
GLPVCGETCAGGTCNTPGCTCSWPVCTRN

SEQ ID NO: 10 - protein, 29 aa, Artificial Sequence
  Mutant form of Kalata B1
GLPVCGETCKGGTCNTPGCTCSWPVCTRN

SEQ ID NO: 11 - DNA, 87 bp, Oldenlandia affinis
ggacttccagtatgcggtgagacttgtgttgggggaacttgcaacactccaggctgcacttgctcctggcctgtttgcacacgcaat

SEQ ID NO: 12 - DNA, 87 bp, Oldenlandia affinis
ggtcttccagtatgcggcgagacttgctttgggggaacttgcaacactccaggctgctcttgcacctggcctatctgcacacgcgat

SEQ ID NO: 13 - protein, 124 aa, Oldenlandia affinis
MAKFTVCLLLCLLLAAFVGAFGSELSDSHKTTLVNEIAEKMLQRKILDGVEATLVTDVAEKMFLRKMKAEAKTSETADQVFLKQLQLKGLPVCGETCVGGTCNTPGCTCSWPVCTRNGLPSLAA

SEQ ID NO: 14 - protein, 210 aa, Oldenlandia affinis
MAKFTNCLVLSLLLAAFVGAFGAEFSEADKATLVNDIAENIQKEILGEVKTSETVLTMFLKEMQLKGLPVCGETCFGGTCNTPGCSCTWPICTRDSLPMRAGGKTSETTLHMFLKEMQLKGLPVCGETCFGGTCNTPGCSCTWPICTRDSLPMSAGGKTSETTLHMFLKEMQLKGLPVCGETCFGGTCNTPGCSCTWPICTRDSLPLVAA

SEQ ID NO: 15 - DNA, 724 bp, Oldenlandia affinis
ggcaccagcactttcttaaaatttactgctttttcttatttcttgttctgtgcttgcttcttccatggctaagttcaccgtctgtctcctcctgtgcttgcttcttgcagcatttgttggggcgtttggatctgagctttctgactcccacaagaccaccttggtcaatgaaatcgctgagaagatgctacaaagaaagatattggatggagtggaagctactttggtcactgatgtcgccgagaagatgttcctaagaaagatgaaggctgaagcgaaaacttctgaaaccgccgatcaggtgttcctgaaacagttgcagctcaaaggacttccagtatgcggtgagacttgtgttgggggaacttgcaacactccaggctgcacttgctcctggcctgtttgcacacgcaatggccttcctagtttggccgcataatttgcttgatcaaactgcaaaaatgaatgagaaggccgacaccaataaagctatcaatgtagttggtccctgtacttaatttggttggctccaaaccatgtgtgctgctcttgtttttgttttttcttttttcttctctctttcgggcactcttcaggacatgaagtgatgatcagtactctttgctatcatgttttctgtgcacaccttctattgtaggtgttgttgtgatgttgatgcccaattggaataaactgttgtcgttgttaaaaaaaaaaaaaaaaa

SEQ ID NO: 16 - DNA, 993 bp, Oldenlandia affinis
ggcaccagatacaacccctttcttataatttattgcttttcttattccttgaaaaaggagaaataatattggatcttccatggctaagttcaccaactgtctcgtcctgagcttgcttctagcagcatttgttggggctttcggagctgagttttctgaagccgacaaggccaccttggtcaatgatatcgctgagaatatccaaaaagagatactgggcgaagtgaagacttctgaaaccgtccttacgatgttcctgaaagagatgcagctcaaaggtcttccagtatgcggcgagacttgctttgggggaacttgcaacactccaggctgctcttgcacctggcctatctgcacacgcgatagccttcctatgagggctggaggaaaaacatctgaaaccacccttcatatgttcctgaaagagatgcagctcaagggtcttccagtttgcggcgagacttgctttgggggaacttgcaacactccaggctgctcgtgcacctggcctatctgcacacgcgatagccttcctatgagtgctggaggaaaaacatctgaaaccacccttcatatgttcctgaaagagatgcagctcaagggtcttccagtttgcggcgagacttgctttgggggaacttgcaacactccaggctgctcgtgcacctggcctatatgcacacgtgatagccttcctcttgtggctgcataatttgcttcatcaaactgcaaaatgaataagaagggacactaaattagctatgaattttgttggcccttgtgtctggtaatttggttcccgccaaattaaccatatgtatgcattgctccttttttctttcttttttttccccctcatttgggcactcttcattacatgaagagatcatgacgctttgttactctgagcaccccctgttggtgttgttcacatgttgatgcccatgttggaataaactcttgtttttgttaccaaaaaaaaaaaaaaaaaaa

SEQ ID NO: 17 - protein, 29 aa, Artificial Sequence
  Mutant form of Kalata B1
  variant 1: Xaa can be any amino acid
  variant 8: /replace="Ala" /replace="Cys" /replace="Asp" /replace="Glu" /replace="Phe" /replace="Gly" /replace="His" /replace="Ile" /replace="Leu" /replace="Met" /replace="Asn" /replace="Pro" /replace="Gln" /replace="Arg" /replace="Ser" /replace="Thr" /replace="Val" /replace="Trp" /replace="Tyr"
  variant 10: /replace="Cys" /replace="Asp" /replace="Glu" /replace="Phe" /replace="Gly" /replace="His" /replace="Ile" /replace="Leu" /replace="Met" /replace="Asn" /replace="Pro" /replace="Gln" /replace="Arg" /replace="Ser" /replace="Thr" /replace="Val" /replace="Trp" /replace="Tyr"
  variant 18: Xaa can be any amino acid
  variant 20: Xaa can be any amino acid
  variant 22: Xaa can be any amino acid
  variant 25: Xaa can be any amino acid
  variant 29: Xaa can be any amino acid
XLPVCGEXCXGGTCNTPXCXCXWPXCTRX